European Patent Specification EP 3 503 880 B1, published December 27, 2023. Title: Compounds for treatment of intractable epilepsy and DOORS syndrome. Applicant: VIB VZW KATHOLIEKE UNIVERSITEIT LEUVEN, K.U.LEUVEN R&D VRIJE UNIVERSITEIT BRUSSEL. The sequence listing filed with the application follows.

SEQUENCE LISTING (5 sequences)

SEQ ID NO: 1 - protein, 346 aa, Homo sapiens
SKPKKIRVCVGTWNVNGGKQFRSIAFKNQTLTDWLLDAPKLAGIQEFQDKRSKPTDIFAIGFEEMVELNAGNIVSASTTNQKLWAVELQKTISRDNKYVLLASEQLVGVCLFVFIRPQHAPFIRDVAVDTVKTGMGGATGNKGAVAIRMLFHTTSLCFVCSHFAAGQSQVKERNEDFIEIARKLSFPMGRMLFSHDYVFWCGDFNYRIDLPNEEVKELIRQQNWDSLIAGDQLINQKNAGQVFRGFLEGKVTFAPTYKYDLFSDDYDTSEKCRTPAWTDRVLWRRRKWPFDRSAEDLDLLNASFQDESKILYTWTPGTLLHYGRAELKTSDHRPVVALIDIDIFEV

SEQ ID NO: 2 - protein, 1311 aa, Homo sapiens
MAFSKGFRIYHKLDPPPFSLIVETRHKEECLMFESGAVAVLSSAEKEAIKGTYSKVLDAYGLLGVLRLNLGDTMLHYLVLVTGCMSVGKIQESEVFRVTSTEFISLRIDSSDEDRISEVRKVLNSGNFYFAWSASGISLDLSLNAHRSMQEQTTDNRFFWNQSLHLHLKHYGVNCDDWLLRLMCGGVEIRTIYAAHKQAKACLISRLSCERAGTRFNVRGTNDDGHVANFVETEQVVYLDDSVSSFIQIRGSVPLFWEQPGLQVGSHRVRMSRGFEANAPAFDRHFRTLKNLYGRQIIVNLLGSKEGEHMLSKAFQSHLKASEHAADIQMVNFDYHQMVKGGKAEKLHSVLKPQVQKFLDYGFFYFNGSEVQRCQSGTVRTNSLDCLDRTNSVQAFLGLEMLAKQLEALGLAEKPQLVTRFQEVFRSMWSVNGDSISKIYAGTGALEGKAKLKDGARSVTRTIQNNFFDSSKQEAIDVLLLGNTLNSDLADKARALLTTGSLRVSEQTLQSASSKVLKSMCENFYKYSKPKKIRVCVGTWNVNGGKQFRSIAFKNQTLTDWLLDAPKLAGIQEFQDKRSKPTDIFAIGFEEMVELNAGNIVSASTTNQKLWAVELQKTISRDNKYVLLASEQLVGVCLFVFIRPQHAPFIRDVAVDTVKTGMGGATGNKGAVAIRMLFHTTSLCFVCSHFAAGQSQVKERNEDFIEIARKLSFPMGRMLFSHDYVFWCGDFNYRIDLPNEEVKELIRQQNWDSLIAGDQLINQKNAGQVFRGFLEGKVTFAPTYKYDLFSDDYDTSEKCRTPAWTDRVLWRRRKWPFDRSAEDLDLLNASFQDESKILYTWTPGTLLHYGRAELKTSDHRPVVALIDIDIFEVEAEERQNIYKEVIAVQGPPDGTVLVSIKSSLPENNFFDDALIDELLQQFASFGEVILIRFVEDKMWVTFLEGSSALNVLSLNGKELLNRTITIALKSPDWIKNLEEEMSLEKISIALPSSTSSTLLGEDAEVAADFDMEGDVDDYSAEVEELLPQHLQPSSSSGLGTSPSSSPRTSPCQSPTISEGPVPSLPIRPSRAPSRTPGPPSAQSSPIDAQPATPLPQKDPAQPLEPKRPPPPRPVAPPTRPAPPQRPPPPSGARSPAPTRKEFGGIGAPPSPGVARREMEAPKSPGTTRKDNIGRSQPSPQAGLAGPGPAGYSTARPTIPPRAGVISAPQSHARASAGRLTPESQSKTSETSKGSTFLPEPLKPQAAFPPQSSLPPPAQRLQEPLVPVAAPMPQSGPQPNLETPPQPPPRSRSSHSLPSEASSQPQQEQPSG

SEQ ID NO: 3 - protein, 1311 aa, Homo sapiens [sequence omitted]

SEQ ID NO: 4 - DNA, 27 bp, Artificial Sequence
  Primer
agaattcatgccataccatcgaggcgg

SEQ ID NO: 5 - DNA, 32 bp, Artificial Sequence
  Primer
aagcggccgcttagatgcccacgaatccgtag